European Patent Specification EP 3 383 377 B1, published April 17, 2024. Title: COMPOUNDS AND METHODS FOR INHIBITING PRODUCTION OF TRIMETHYLAMINE. Applicant: The Procter & Gamble Company. The sequence listing filed with the application follows.

SEQUENCE LISTING (5 sequences)

SEQ ID NO: 1 - DNA, 2146 bp, Escherichia coli
atgagcaatctgagccctgactttgtactacccgaaaatttttgcgctaacccgcaagaggcgtggaccattcctgcccgtttttataccgatcagaacgcgtttgaacacgaaaaagagaacgtcttcgccaaaagctggatttgcgtcgctcacagcagcgaactggcgaatgccaatgattatgtgacgcgtgagatcattggcgaaagcatcgtgctggtacgcggtcgtgataaggttttgcgcgcgttctataacgtgtgtccgcaccgtggtcatcagttgttgagcggtgaaggaaaagcaaaaaatgtgattacctgcccgtatcacgcatgggcattcaaactcgatggcaacctggcccatgcacgtaactgcgaaaacgtcgccaatttcgatagcgacaaagcgcaactggttccggtgcgtctggaagaatatgccggattcgtcttcatcaacatggaccccaacgccaccagcgtagaagatcaattacccggcctgggcgcgaaagtgctggaagcctgcccggaagtccacgatctgaaactggcggcccgctttaccacccgcacgcctgccaactggaagaacattgtcgataactatctcgagtgctatcactgtggtccggcgcatccaggtttctccgactccgtacaggttgatcgttactggcacaccatgcacggtaactggacgctgcaatacggtttcgccaaaccgtccgaacagtcgtttaaatttgaagagggtacggatgcggcattccacggtttctggctgtggccgtgcacgatgctgaacgtcaccccgatcaaagggatgatgacggtcatttatgaattcccggtggattctgaaactaccctgcaaaactacgatatttacttcaccaatgaagagttaaccgacgagcaaaaatcgctgattgagtggtatcgcgatgtgttccgtccggaagatttacgtctggttgaaagcgtacagaaagggctgaaatcgcgtggctatcgtggtcaggggcgcatcatggccgacagtagcggtagtggcatttccgaacatggtatcgcccatttccataatctgctggcgcaggtgtttaaggactaatgacatcggcggcggtattttccgccgctgggctgatttttgatggagtacagcaatgtcagactatcaaatgtttgaagtacaggtgagccaggttgaaccccttaccgaacaggtgaaacgcttcacgctggtggcaaccgatggcaaaccattacctgcgtttaccggaggaagtcacgtcattgtgcagatgagcgatggtgataaccagtacagcaatgcgtattcactactgagttcgccgcatgacacctcttgttatcagattgccgttcggctggaggaaaactcgcgcggcggttcccgctttttgcatcagcaggtaaaagtgggcgatcggttaacgatttcaacgcctaataacctgtttgcgctaattccctcagccagaaagcatctgtttatcgcgggcggtattggtatcacccctttcctgtcgcacatggcagagctgcaacacagcgacgtcgactggcagctacattactgctcgcgaaatccagaaagttgcgcatttcgtgatgagctagtccagcatccgcaggctgagaaagtccatttgcatcattcatcaaccggaacacgactggaattagcgcgattattggcggatatcgaacctggcacacacgtttatacctgtggccccgaggcgctaattgaagcggtaagaagtgaagctgcgcgtctggacatcgccgccgatacgctgcactttgagcaatttgctatcgaagacaaaaccggcgatgcatttaccctggtgcttgcccgttccggaaaagagtttgtggtgccggaagagatgactattttgcaggttattgaaaataataaagccgcgaaagtggaatgtttatgtcgtgaaggggtatgcggaacctgcgaaacagcaatactggaaggtgaagctgaccatcgggatcaatattttagcgatgaagagcgtgccagccagcaaagtatgttgatctgttgttcgcgtgcgaagggtaaacgcctggtgttggatttgtag

SEQ ID NO: 2 - protein, 374 aa, Escherichia coli
MSNLSPDFVLPENFCANPQEAWTIPARFYTDQNAFEHEKENVFAKSWICVAHSSELANANDYVTREIIGESIVLVRGRDKVLRAFYNVCPHRGHQLLSGEGKAKNVITCPYHAWAFKLDGNLAHARNCENVANFDSDKAQLVPVRLEEYAGFVFINMDPNATSVEDQLPGLGAKVLEACPEVHDLKLAARFTTRTPANWKNIVDNYLECYHCGPAHPGFSDSVQVDRYWHTMHGNWTLQYGFAKPSEQSFKFEEGTDAAFHGFWLWPCTMLNVTPIKGMMTVIYEFPVDSETTLQNYDIYFTNEELTDEQKSLIEWYRDVFRPEDLRLVESVQKGLKSRGYRGQGRIMADSSGSGISEHGIAHFHNLLAQVFKD

SEQ ID NO: 3 - protein, 321 aa, Escherichia coli
MSDYQMFEVQVSQVEPLTEQVKRFTLVATDGKPLPAFTGGSHVIVQMSDGDNQYSNAYSLLSSPHDTSCYQIAVRLEENSRGGSRFLHQQVKVGDRLTISTPNNLFALIPSARKHLFIAGGIGITPFLSHMAELQHSDVDWQLHYCSRNPESCAFRDELVQHPQAEKVHLHHSSTGTRLELARLLADIEPGTHVYTCGPEALIEAVRSEAARLDIAADTLHFEQFAIEDKTGDAFTLVLARSGKEFVVPEEMTILQVIENNKAAKVECLCREGVCGTCETAILEGEADHRDQYFSDEERASQQSMLICCSRAKGKRLVLDL

SEQ ID NO: 4 - DNA, 33 bp, Escherichia coli
catgccatatgagcaatctgagccctgactttg

SEQ ID NO: 5 - DNA, 38 bp, Escherichia coli
catactgcagctacaaatccaacaccaggcgtttaccc